European Patent Specification EP 4 168 013 B1, published October 22, 2025. Title: Method for treatement of pancreatitis. Applicant: NovMetaHealth Co., Ltd. The sequence listing filed with the application follows.

SEQUENCE LISTING (6 sequences)

SEQ ID NO: 1 - DNA, 20 bp, artificial sequence
  Esrra forward primer
tacggtgtggcatcctgtga

SEQ ID NO: 2 - DNA, 20 bp, Artificial Sequence
  Essr reverse primer
ctcccctggatggtcctctt

SEQ ID NO: 3 - DNA, 18 bp, Artificial sequence
  Esrrg forward primer
gcccagccacgaatgaat

SEQ ID NO: 4 - DNA, 18 bp, Artificial sequence
  Esrrg reverse primer
gcaggcctggcaggattt

SEQ ID NO: 5 - DNA, 20 bp, Artificial sequence
  36b4 forward primer
acctccttcttccaggcttt

SEQ ID NO: 6 - DNA, 20 bp, Artificial sequence
  3664 reverse primer
ctccagtctttatcagctgc